European Patent Application EP 4 357 360 A1, published April 24, 2024. Title: A human antibody against the receptor- binding motif on the preS1 of hepatitis B Virus and an use thereof. Applicant: APITBIO, Inc. The sequence listing filed with the application follows.

SEQUENCE LISTING (19 sequences)

SEQ ID NO: 1 - protein, 107 aa, Artificial Sequence
  Light chain
  MISC_FEATURE (24)..(34): LCDR1
  MISC_FEATURE (50)..(56): LCDR2
  MISC_FEATURE (89)..(97): LCDR3, X can be any amino acid
DIQMTQSPSSLSASVGDRVTITCRASQSIASYLNWYQQKPGKAPKLLIYATSRLQSGVPSRFSGSGSGTDFTLTISSLQPEDFATYYCQQXXXXPYTFGQGTKVEIK

SEQ ID NO: 2 - protein, 117 aa, Artificial Sequence
  Heavy chain
  MISC_FEATURE (31)..(35): HCDR1
  MISC_FEATURE (33): X can be any amino acid (preferably S, P, V or A)
  MISC_FEATURE (50)..(66): HCDR2
  MISC_FEATURE (50): X is Ser or Ala
  MISC_FEATURE (53): X can be any amino acid
  MISC_FEATURE (99)..(106): HCDR3, X can be any amino acid
EVQLVESGGGLVQPGGSLRLSCAASGFTFSTYXMSWVRQAPGKGLEWVSXISQSGGYTNYADSVKGRFTISRDNSKNTLYLQMNSLRAEDTAVYYCAKVIYASLDYWGQGTLVTVSS

SEQ ID NO: 3 - protein, 11 aa, Artificial Sequence
  Light chain CDR1 (LCDR1)
RASQSIASYLN

SEQ ID NO: 4 - protein, 7 aa, Artificial Sequence
  Light chain CDR2 (LCDR2)
ATSRLQS

SEQ ID NO: 5 - protein, 9 aa, Artificial Sequence
  Light chain CDR3 (LCDR3)
  MISC_FEATURE (3)..(6): X can be any amino acid
  MISC_FEATURE (8): paratope
QQXXXXPYT

SEQ ID NO: 6 - protein, 9 aa, Artificial Sequence
  LCDR3
QQSYSSPYT

SEQ ID NO: 7 - protein, 5 aa, Artificial Sequence
  HCDR1
  MISC_FEATURE (3): X can be any amino acid (preferably S, P, V or A)
TYXMS

SEQ ID NO: 8 - protein, 17 aa, Artificial Sequence
  HCDR2
  MISC_FEATURE (1): X is Ser or Ala
  MISC_FEATURE (1): paratope
  MISC_FEATURE (4): X can be any amino acid
XISXSGGYTNYADSVKG

SEQ ID NO: 9 - protein, 8 aa, Artificial Sequence
  HCDR3
  MISC_FEATURE (1): X can be any amino acid
  MISC_FEATURE (5): X can be any amino acid
  MISC_FEATURE (6): paratope
XIYAXLDY

SEQ ID NO: 10 - protein, 5 aa, Artificial Sequence
  HCDR1
TYAMS

SEQ ID NO: 11 - protein, 17 aa, Artificial Sequence
  HCDR2_AbS0
  MISC_FEATURE (1): paratope
AISQSGGYTNYADSVKG

SEQ ID NO: 12 - protein, 17 aa, Artificial Sequence
  HCDR2_AbS1
  MISC_FEATURE (1): paratope
SISQSGGYTNYADSVKG

SEQ ID NO: 13 - protein, 8 aa, Artificial Sequence
  HCDR3
VIYASLDY

SEQ ID NO: 14 - protein, 107 aa, Artificial Sequence
  Light chain
DIQMTQSPSSLSASVGDRVTITCRASQSIASYLNWYQQKPGKAPKLLIYATSRLQSGVPSRFSGSGSGTDFTLTISSLQPEDFATYYCQQSYSSPYTFGQGTKVEIK

SEQ ID NO: 15 - protein, 117 aa, Artificial Sequence
  Heavy chain_AbS0
EVQLVESGGGLVQPGGSLRLSCAASGFTFSTYAMSWVRQAPGKGLEWVSAISQSGGYTNYADSVKGRFTISRDNSKNTLYLQMNSLRAEDTAVYYCAKVIYASLDYWGQGTLVTVSS

SEQ ID NO: 16 - protein, 117 aa, Artificial Sequence
  Heavy chain_AbS1
EVQLVESGGGLVQPGGSLRLSCAASGFTFSTYAMSWVRQAPGKGLEWVSSISQSGGYTNYADSVKGRFTISRDNSKNTLYLQMNSLRAEDTAVYYCAKVIYASLDYWGQGTLVTVSS

SEQ ID NO: 17 - protein, 7 aa, Artificial Sequence
  preS1_epitope 1
NPLGFFP

SEQ ID NO: 18 - protein, 7 aa, Artificial Sequence
  preS1_epitope 2
NPLGFLP

SEQ ID NO: 19 - protein, 119 aa, Artificial Sequence
  preS1
  MISC_FEATURE (20)..(26): receptor binding motif
MGGWSSKPRQGMGTNLSVPNPLGFFPDHQLDPAFGANSNNPDWDFNPNKDHWPDGNQVGVGAFGPGFTPPHGGLLGWSPQAQGILTTVPAAPPPASTNRQSGRQPTPISPPLRDSHPQA